European Patent Application EP 4 656 735 A1, published December 3, 2025. Title: リボソーマルＲＮＡ由来の逆転写の抑制. Applicant: 東洋紡株式会社. The sequence listing filed with the application follows.

SEQUENCE LISTING (4 sequences)

SEQ ID NO: 1 - DNA, 20 bp, synthetic construct
  source 1..20: mol_type = other DNA; note = forward primer
cgcgagaagatgacccagat

SEQ ID NO: 2 - DNA, 20 bp, synthetic construct
  source 1..20: mol_type = other DNA; note = reverse primer
gccagaggcgtacagggata

SEQ ID NO: 3 - DNA, 18 bp, synthetic construct
  source 1..18: mol_type = other DNA; note = forward primer
gatggtagtcgccgtgcc

SEQ ID NO: 4 - DNA, 18 bp, synthetic construct
  source 1..18: mol_type = other DNA; note = reverse primer
gcctgctgccttccttgg